European Patent Application EP 4 682 269 A1, published January 21, 2026. Title: Method for amplification of complementary DNA strands. Applicant: イムノジェネテクス株式会社. Application JP. The sequence listing filed with the application follows.

SEQUENCE LISTING (41 sequences)

SEQ ID NO: 1 - DNA, 89 bp, synthetic construct
  source 1..89: mol_type = other DNA
  misc_feature 21: note = n is none or A or GT or TCA.
  misc_feature 22..30: note = CLS1
  misc_feature 35..43: note = CLS2
  misc_feature 48..56: note = CLS3
  misc_feature 57..64: note = n is A, T, C or G.
acacgacgctcttccgatctnnnnnnnnnngtgannnnnnnnngacannnnnnnnnnnnnnnnnttttttttttttttttttttttttt

SEQ ID NO: 2 - DNA, 33 bp, synthetic construct
  source 1..33: mol_type = other DNA
acactctttccctacacgacgctcttccgatct

SEQ ID NO: 3 - DNA, 28 bp, synthetic construct
  misc_feature 26..28: note = RNA
  source 1..28: mol_type = other DNA
aagcagtggtatcaacgcagagtacggg

SEQ ID NO: 4 - DNA, 22 bp, synthetic construct
  source 1..22: mol_type = other DNA
aagcagtggtatcaacgcagag

SEQ ID NO: 5 - DNA, 82 bp, synthetic construct
  source 1..82: mol_type = other DNA
  misc_feature 23..38: note = CB
  misc_feature 39..50: note = n is A, T, C or G.
  misc_feature 81: note = v is A, G or C.
  misc_feature 82: note = n is A, T, C or G.
ctacacgacgctcttccgatctnnnnnnnnnnnnnnnnnnnnnnnnnnnnttttttttttttttttttttttttttttttvn

SEQ ID NO: 6 - DNA, 30 bp, synthetic construct
  misc_feature 28..30: note = RNA
  source 1..30: mol_type = other DNA
aagcagtggtatcaacgcagagtacatggg

SEQ ID NO: 7 - DNA, 50 bp, synthetic construct
  source 1..50: mol_type = other DNA
aagcagtggtatcaacgcagagtacttttttttttttttttttttttttt

SEQ ID NO: 8 - DNA, 28 bp, synthetic construct
  misc_feature 26..28: note = RNA
  source 1..28: mol_type = other DNA
aagcagtggtatcaacgcagagtacggg

SEQ ID NO: 9 - DNA, 23 bp, synthetic construct
  source 1..23: mol_type = other DNA
aagcagtggtatcaacgcagagt

SEQ ID NO: 10 - DNA, 33 bp, synthetic construct
  source 1..33: mol_type = other DNA
gatcggaagagcacacgtctgaactccagtcac

SEQ ID NO: 11 - DNA, 13 bp, synthetic construct
  source 1..13: mol_type = other DNA
gctcttccgatct

SEQ ID NO: 12 - DNA, 57 bp, synthetic construct
  source 1..57: mol_type = other DNA
aatgatacggcgaccaccgagatctacacatccatatacactctttccctacacgac

SEQ ID NO: 13 - DNA, 57 bp, synthetic construct
  source 1..57: mol_type = other DNA
aatgatacggcgaccaccgagatctacacgcttgcgcacactctttccctacacgac

SEQ ID NO: 14 - DNA, 57 bp, synthetic construct
  source 1..57: mol_type = other DNA
aatgatacggcgaccaccgagatctacacagtatcttacactctttccctacacgac

SEQ ID NO: 15 - DNA, 57 bp, synthetic construct
  source 1..57: mol_type = other DNA
aatgatacggcgaccaccgagatctacacattggaacacactctttccctacacgac

SEQ ID NO: 16 - DNA, 57 bp, synthetic construct
  source 1..57: mol_type = other DNA
aatgatacggcgaccaccgagatctacacgccaaggtacactctttccctacacgac

SEQ ID NO: 17 - DNA, 57 bp, synthetic construct
  source 1..57: mol_type = other DNA
aatgatacggcgaccaccgagatctacaccgagatatacactctttccctacacgac

SEQ ID NO: 18 - DNA, 57 bp, synthetic construct
  source 1..57: mol_type = other DNA
aatgatacggcgaccaccgagatctacacttcacaatacactctttccctacacgac

SEQ ID NO: 19 - DNA, 57 bp, synthetic construct
  source 1..57: mol_type = other DNA
aatgatacggcgaccaccgagatctacacacacgagtacactctttccctacacgac

SEQ ID NO: 20 - DNA, 57 bp, synthetic construct
  source 1..57: mol_type = other DNA
aatgatacggcgaccaccgagatctacacgtgtagacacactctttccctacacgac

SEQ ID NO: 21 - DNA, 53 bp, synthetic construct
  source 1..53: mol_type = other DNA
caagcagaagacggcatacgagatcttagtgtgtgactggagttcagacgtgt

SEQ ID NO: 22 - DNA, 53 bp, synthetic construct
  source 1..53: mol_type = other DNA
caagcagaagacggcatacgagattccgacacgtgactggagttcagacgtgt

SEQ ID NO: 23 - DNA, 53 bp, synthetic construct
  source 1..53: mol_type = other DNA
caagcagaagacggcatacgagataacaggaagtgactggagttcagacgtgt

SEQ ID NO: 24 - DNA, 53 bp, synthetic construct
  source 1..53: mol_type = other DNA
caagcagaagacggcatacgagatacacgagtgtgactggagttcagacgtgt

SEQ ID NO: 25 - DNA, 53 bp, synthetic construct
  source 1..53: mol_type = other DNA
caagcagaagacggcatacgagatgtgtagacgtgactggagttcagacgtgt

SEQ ID NO: 26 - DNA, 53 bp, synthetic construct
  source 1..53: mol_type = other DNA
caagcagaagacggcatacgagatgttaattggtgactggagttcagacgtgt

SEQ ID NO: 27 - DNA, 53 bp, synthetic construct
  source 1..53: mol_type = other DNA
caagcagaagacggcatacgagatcgcagacggtgactggagttcagacgtgt

SEQ ID NO: 28 - DNA, 53 bp, synthetic construct
  source 1..53: mol_type = other DNA
caagcagaagacggcatacgagatgatatcgagtgactggagttcagacgtgt

SEQ ID NO: 29 - DNA, 53 bp, synthetic construct
  source 1..53: mol_type = other DNA
caagcagaagacggcatacgagatagcgctaggtgactggagttcagacgtgt

SEQ ID NO: 30 - DNA, 57 bp, synthetic construct
  source 1..57: mol_type = other DNA
aatgatacggcgaccaccgagatctacacgtctcgcaacactctttccctacacgac

SEQ ID NO: 31 - DNA, 57 bp, synthetic construct
  source 1..57: mol_type = other DNA
aatgatacggcgaccaccgagatctacacaagacgtcacactctttccctacacgac

SEQ ID NO: 32 - DNA, 57 bp, synthetic construct
  source 1..57: mol_type = other DNA
aatgatacggcgaccaccgagatctacacggagtactacactctttccctacacgac

SEQ ID NO: 33 - DNA, 57 bp, synthetic construct
  source 1..57: mol_type = other DNA
aatgatacggcgaccaccgagatctacaccactacgaacactctttccctacacgac

SEQ ID NO: 34 - DNA, 57 bp, synthetic construct
  source 1..57: mol_type = other DNA
aatgatacggcgaccaccgagatctacactgtcgtagacactctttccctacacgac

SEQ ID NO: 35 - DNA, 57 bp, synthetic construct
  source 1..57: mol_type = other DNA
aatgatacggcgaccaccgagatctacacaccacttaacactctttccctacacgac

SEQ ID NO: 36 - DNA, 53 bp, synthetic construct
  source 1..53: mol_type = other DNA
caagcagaagacggcatacgagatgtccgtgcgtgactggagttcagacgtgt

SEQ ID NO: 37 - DNA, 53 bp, synthetic construct
  source 1..53: mol_type = other DNA
caagcagaagacggcatacgagataaggtaccgtgactggagttcagacgtgt

SEQ ID NO: 38 - DNA, 53 bp, synthetic construct
  source 1..53: mol_type = other DNA
caagcagaagacggcatacgagatggaacgttgtgactggagttcagacgtgt

SEQ ID NO: 39 - DNA, 53 bp, synthetic construct
  source 1..53: mol_type = other DNA
caagcagaagacggcatacgagatcagttccggtgactggagttcagacgtgt

SEQ ID NO: 40 - DNA, 53 bp, synthetic construct
  source 1..53: mol_type = other DNA
caagcagaagacggcatacgagattgaccttagtgactggagttcagacgtgt

SEQ ID NO: 41 - DNA, 53 bp, synthetic construct
  source 1..53: mol_type = other DNA
caagcagaagacggcatacgagatctaggcaagtgactggagttcagacgtgt